European Patent Application EP 4 725 302 A2, published April 15, 2026. Title: COMPOSITIONS AND METHODS FOR PRODUCING PEA PLANTS WITH ENHANCED YIELD, HEIGHT, AND/OR LODGING PHENOTYPE. Applicant: Confluence Genetics, LLC. The sequence listing filed with the application follows.

SEQUENCE LISTING (124 sequences)

SEQ ID NO: 1 - DNA, 201 bp, Pisum sativum
  source 1..201: mol_type = genomic DNA
  variation 101: note = n = t or c
cataatttcgacacccactgtagaattaccaaaatagaaatcctatgtagagatgtttcaaccatgaagagatgtttcgatcgagtagatacgtttcggcnggatatgatattaaagagacccagtcgaaagtccctgggtaataagggtcatcgtgtagttaagacttagaaatatttcttcaaatggttgaagacgact

SEQ ID NO: 2 - DNA, 201 bp, Pisum sativum
  source 1..201: mol_type = genomic DNA
  variation 101: note = n = a or t
ggatttcagctctctgacccttctctcatgggaaagtattttagcaaacctacaaagattaaaaagcagttaaaaaaaatataacttgtattttcaagaangctaacttgtgttttagggagaagttgaaaaacttaataccttttgagagcctcttcatttgtttctccgttttcaattggctcaaacacattggtcttt

SEQ ID NO: 3 - DNA, 201 bp, Pisum sativum
  source 1..201: mol_type = genomic DNA
  variation 101: note = c or t
attattaataacttgtttaattaaaataactaaacatgtgttttttggattctaagagtattatatataaaataatttcattttcaagttttttcttactntgaaatcctatgtacaaatagagtacatccgaaaggatttattgtagaaggaattttgactaatgaatgtttgatattttattcacaaaatttatctgga

SEQ ID NO: 4 - DNA, 201 bp, Pisum sativum
  source 1..201: mol_type = genomic DNA
  variation 101: note = c or t
attttgttgttgattctgcggaggcggtgttataggttgttgatcttgatgcttgaaatacgccaattatggatactgattaggatttaccgtagccacanaagggttgtaaggcccctgggaatatccatcaatagtaacaacattggcatcaaccttctttgaattactattgttaggatactttttgttgttgtgttg

SEQ ID NO: 5 - DNA, 201 bp, Pisum sativum
  source 1..201: mol_type = genomic DNA
  variation 101: note = n = g or a
tattatttgtttatttatattttcttgggtgatctttgtgttaagataagtcctaacccggactttagtgcatattgagataggagggtggtatagtcaanttggcttgggtggaataatcccgaataagatgacttgagaatcccccaatcagtggaggcccctttggggatagtatttgttgaacgagcaatcgtgaag

SEQ ID NO: 6 - DNA, 201 bp, Pisum sativum
  source 1..201: mol_type = genomic DNA
  variation 101: note = n = g or c
aactaataaatagtgtgtatgaactatattcgaagatccatttctgaattataaaaatatttttgtttttcacgaaggtgaggaagaaatctttatagtgngttaaaataaggagatttttgaatgcatccgatatgtttcttaaccatcacacaaaaatactaaaatactctttagatttgggagattcatatctgaaag

SEQ ID NO: 7 - DNA, 201 bp, Pisum sativum
  source 1..201: mol_type = genomic DNA
  variation 101: note = n = t or c
acattaggcgcccaccgtggctctccaataaaaatttcatgggctacaagaatctttctgaacaattggtcccacccttccatgacagaactagcaatagnagtcaagggtcacatgttgtcgttatggagttactctcagtcacgaaagacctcttccatcaaaataaattattgtaggacaatgtgttggtcttacaac

SEQ ID NO: 8 - DNA, 201 bp, Pisum sativum
  source 1..201: mol_type = genomic DNA
  variation 101: note = n = a or g
ttagagaaggtgatcttgtgctcaagaagattctgtctttcaaaccagattctaggggaaaatggactcctaattatgaaggcccatacgttgttaaaagngctttttcaggcggcactttgattcttacaactatggatggtgaagagttcactcgtcctgtgaatgctgatgcattcaagaaatctaattatgttcctc

SEQ ID NO: 9 - DNA, 201 bp, Pisum sativum
  source 1..201: mol_type = genomic DNA
  variation 101: note = n = g or a
ttcaatatcgacataacttctaaacactctactacttctactatttcagatgctcttctagtctctgatgcaacatctgatcagaaggtcagaccttctgnaggcattccttcaacctttctttcttaggcactgaagccacagaagaagattagtagaaagaagaagaagaagaagaagtccaagaggagatacgaagaa

SEQ ID NO: 10 - DNA, 201 bp, Pisum sativum
  source 1..201: mol_type = genomic DNA
  variation 101: note = n = c or t
ttgcacatttctacgagaaataatgaattaagaatgaatttatatcctctatgcaccttagaataatgaaattgttgaggaagaacataaacatactaaanataactagaagcgggcttaaagaaaagaagatgttgtataaattatgaggtgtagcagttacaacatttatgcatattttcaacaagaatctgacaaata

SEQ ID NO: 11 - DNA, 201 bp, Pisum sativum
  source 1..201: mol_type = genomic DNA
  variation 101: note = n = c or t
ccaaagtcaaattttggggtgcgacacttagtagttgaagcagaaagcgatggcaaaccatggttttgatatcaagcgatatcttgagaagcacgagtatncagatgacgtctccatcacagacaagaagaccttgagggagttatcagctaatttatttctaattggtggtgtgctatacaaaagaaattttaatatggg

SEQ ID NO: 12 - DNA, 201 bp, Pisum sativum
  source 1..201: mol_type = genomic DNA
  variation 101: note = n = g or a
tatttcttaatcaaatgcttcaaaacacttaagcatattcaaagatctttacataagacctaaaaaacacaaacttaattcaaacccttttgctactttgntttttccatgtttaaaaccttttcataaaatgattggacatgagttatccctagttgagatttaaatcttctaccccataatattgttgagattgatatt

SEQ ID NO: 13 - DNA, 201 bp, Pisum sativum
  source 1..201: mol_type = genomic DNA
  variation 101: note = n = a or g
ctgactatcatgtcttgtagatatttgccaaatctcgacgtaacttccttagatcaactaaattatagagatttatcgacgtgattgcttcaaattgactngaaattgaagtgtcttgtctttctgctcaatgaatttcttatacgttcaacttcttgatatgatcaaatgaaatgacttgcccctgctcaacggagtctc

SEQ ID NO: 14 - DNA, 201 bp, Pisum sativum
  source 1..201: mol_type = genomic DNA
  variation 101: note = n =g or a
tgtgtggatagacacgaagcagacttattgatgactgaagtccatgaaggttcctttggtactcactccaatggacatgttatggcaaagaagatgttganagcaggttactattggatgacaatggaatctgactgttgcaagtttgtgaagaaatcccacaagtgtcaaatttatgcagataagattcatgttcctccg

SEQ ID NO: 15 - DNA, 201 bp, Pisum sativum
  source 1..201: mol_type = genomic DNA
  variation 101: note = n = t or g
gagaatacttggttgaaatgaaattggaaggtacatttagttagagtttggttactttatacacaaagtacccttaaaatggtgaggtgtcaaacaaagancaaagagtgtttttggattttccaaagcattgtattttcttatatggtagataggtacstacrraaaaaaattgtttgaagaagtggaaaaaatgatata

SEQ ID NO: 16 - DNA, 201 bp, Pisum sativum
  source 1..201: mol_type = genomic DNA
  variation 101: note = n = t or c
crgaktrrcggatgctgataccarcacttgtgattacgtttaaattattaattttttcaaattattaccggtgtcgccatgtcaatgtcggtgttgtgttngtgtgtctgtgcttcataggttgatttcattttcattattgataagcagaatatmtgacaatgttgttcagcgggaaatgtttaaatcamgtcattagtt

SEQ ID NO: 17 - DNA, 201 bp, Pisum sativum
  source 1..201: mol_type = genomic DNA
  variation 101: note = n = c or t
tgtcattcayactctcattaactagtatatcatatttgaactttttaggcatgtatcttgtagattctttaattagtggcttatcaatattgttgtctttnaacttctaaaatttatcaatattatgaccccaaaaaaagaggtaaactatcatattccttcaacaaagaatgtataaccctcttgttccactaaaatacg

SEQ ID NO: 18 - DNA, 201 bp, Pisum sativum
  source 1..201: mol_type = genomic DNA
  variation 101: note = n = g or a
aatccttctagataatgagattaattgttatacactgtcagtgtaaaaagttttacaccgtcaatgcatcacaatcatccgtttgtattactttttaaatngttgaaataaaagtcaaacattttaaataaatcaatggttgtgattaactgacagtgtaaaatctctttacactgtyagtgtatttcaattaaatccttc

SEQ ID NO: 19 - DNA, 201 bp, Pisum sativum
  source 1..201: mol_type = genomic DNA
  variation 101: note = n = g or t
agattcaatgaagattgaacattgttggggatgacaccaataccacaggacccrsrgggaacaaaattyacttmtgactgcttgrggaataacttatcacntctttckcykgggatgacagagtcttgcattgtcgggrataagaggaytcatgcacagaattctggctrgggatgaagtaatsttcaaaactacacttct

SEQ ID NO: 20 - DNA, 201 bp, Pisum sativum
  source 1..201: mol_type = genomic DNA
  variation 101: note = n = g or a
tgttaacaataatcattgggttcaggtaaagttgaaacctgatagtccattgccttccgtcacttaccgttggagacaaaattstactgaagacgcaaaancatgagaatcaacacatatgtaggatgcattaggcactaggaagatgaagttaggaaatcatcctattttgttttgtaatcttgtatgtagtataatttt

SEQ ID NO: 21 - DNA, 201 bp, Pisum sativum
  source 1..201: mol_type = genomic DNA
  variation 101: note = n = c or t
aggtattagcaaccctacgcatycgtcgtactcaacgggatccacgctcaaaaggatagaagaaaggttgctaaacactgctcaaaagaatgcaygcacantggaataaaacacatattraakaagaggggraaacgggctcgctaggatatcgcatcctatrcctacgtatctcatctggaatgagaatcagagctaccg

SEQ ID NO: 22 - DNA, 201 bp, Pisum sativum
  source 1..201: mol_type = genomic DNA
  variation 101: note = n = a or g
tcatttcgtaccatgcttgcatcattttgccaaaattggaaagttgagtgagtgtgcaaatatcwtttgaattctctataaattgaagccctcatgctcanaaatcacaaacaccttacgcyarctttgaatccccacagaaaacccttcacattaagaggataaacctgaaaaattcagttgaatttgagcttgaatctc

SEQ ID NO: 23 - DNA, 201 bp, Pisum sativum
  source 1..201: mol_type = genomic DNA
  variation 101: note = n = c or t
tctcccccctttyatggtattatrtggaaacttsgccttttttccttcctttggaagatgtcttggttcaaggatycatgcttgtgaatagagggttgagngttctccaaagaatgacttaaccaattgaaaagcaaaacaccactaacatctaatcaactaacattttgattaacctatactctttgcttttaatttcaa

SEQ ID NO: 24 - DNA, 201 bp, Pisum sativum
  source 1..201: mol_type = genomic DNA
  variation 101: note = n = a or c
ctcctcataatcaattacacaagtttcataatcgattaaagagtgaacttagatrtataatcaattaactaagcattacaatcaattaagctccatttttnaaaagtttttccmaaaccaagatgtttttagatgttttttttaaaacatatgaaattttaataaattttgtgtatgcaaccatactttgaaagcattcas

SEQ ID NO: 25 - DNA, 201 bp, Pisum sativum
  source 1..201: mol_type = genomic DNA
  variation 101: note = n = g or a
aggrtaattcagtattttagtattttgtctaygtgkcattattctgtgtatataagtagtagtgtgcttagctattaagtaacataacwgtmtgtacacancagagcartgtgagtgcaaccattttgctgtaaytgtttttagcagagtaarggaaatttgttattctctcttctctctyttcttccatcttcatcttct

SEQ ID NO: 26 - DNA, 201 bp, Pisum sativum
  source 1..201: mol_type = genomic DNA
  variation 101: note = n = t or c
taaagcaaagaataaaccaatccctacaagtgaagtccatagtgctatgaaacaagaggtacaataccagaactgctcctcataattcttatgatgcatgntttcctgtaatcatgttatattcatttcactttggcctatttaatcatgttcttttgtttgtctttttctggttggtgcattgcattcatcaatatmtaa

SEQ ID NO: 27 - DNA, 201 bp, Pisum sativum
  source 1..201: mol_type = genomic DNA
  variation 101: note = n = g or a
ttaacaagatgagggatcgttgragctcatggaaggaaattcaaaactaraaaaagagagagtgtttgaacaaagaagcgaaaacattacatgaaaagagnagmcacatttatatagtgggayaaggtaggccaatatacagctcatgacgaaggcaatctaagcagatgaaatcaacaaagagatttaccttgaaatcac

SEQ ID NO: 28 - DNA, 201 bp, Pisum sativum
  source 1..201: mol_type = genomic DNA
  variation 101: note = n =g or a
aaaattatttttaatatgcatgatatcaaagtttataataagcgtgyacctaaaatatatagctmttgttgtttagtcaagtcacatagatttaattttgnrtaggggtgttcatgagtacgggtggatccgtgaayctactgatccaaaytgaatcaaccmataaattatcgaaayccrttyattacaagtatacacaat

SEQ ID NO: 29 - DNA, 201 bp, Pisum sativum
  source 1..201: mol_type = genomic DNA
  variation 101: note = n = a or t
tgtcaagtttttatgtgtgattaagtcttcattatgcatgttagtttaaatcttcrttwagtctttgtctttaaattctatttggtagtaatcctcgagtngtttttatatccggtcaaacaccatctatatgcacacatttgagttrggttggtcgacaaataataagtgaatatcatttgctaataattgaataaaaaa

SEQ ID NO: 30 - DNA, 201 bp, Pisum sativum
  source 1..201: mol_type = genomic DNA
  variation 101: note = n = g or t
tgtccttattcaragatgcattraaaattgttraaragggtcattcagatcggtgggggaaaatggtatasgtctccgwcaacaagagcagagccgrtttnggtttccaacgaggttcaccartggttagatmtgaagatgtgcaacccartttccgtagcggaggkttcattcatagtaatgaacaacacttagytgttg

SEQ ID NO: 31 - DNA, 201 bp, Pisum sativum
  source 1..201: mol_type = genomic DNA
  variation 101: note = n = c or a
attattatcatgtgaggtttgatatataacaggatcttatgctgcttgtcaagaaatttggattagatatgtgaagcaagatatgaatgtcgaagtgaagnaacctttggtgttgcarattaacaacaagtcatctatgaatctcgcaaagaatccaattctacatgggagaagtaagcacatcgagcctaggtttcatgt

SEQ ID NO: 32 - DNA, 201 bp, Pisum sativum
  source 1..201: mol_type = genomic DNA
  variation 101: note = n = a or g
tcatgaagatcaccatgtagaaatacatcatggacatctagccgatgaataggtcgygatttggacagagcaatggtgagaayggagygaatagtggccgntttgaccacatgaccraatgtctcattataatctacacctgaaatatgtgaccttccatcacctacaagaygagctttgtaggctgaaagcaaccattag

SEQ ID NO: 33 - DNA, 201 bp, Pisum sativum
  source 1..201: mol_type = genomic DNA
  variation 101: note = n = a or g
ggcatcgttgaagcakcaaacaagaacatcaagaagatcatccagaaaatggtgataacatataagtattgacatgaaattctactttttgtgttgyacgnctatcgaacgtcagtttgcacttcaacaagggcatcccttactcattagtatatggcatggaagtggtccttctagtagaagttgaaatkccattggtga

SEQ ID NO: 34 - DNA, 201 bp, Pisum sativum
  source 1..201: mol_type = genomic DNA
  variation 101: note = n = a or g
gyrtgtgtayrtgtgctmrttayyratygmctcctaggaaatctcatttaaaagccgtaaaaygcattcttaggtatcttmctggtaattctaagtatgrnytttggtattctawgggaagcgattgtwatttggttggttataycgattcckattttkywgrttgyaaatcakatargaagaatactagtggaacttgtc

SEQ ID NO: 35 - DNA, 201 bp, Pisum sativum
  source 1..201: mol_type = genomic DNA
  variation 101: note = n = t or c
ccccaatcttawtttttyctccgwggcccatgctgaaaaatatctcaaactagtggattaccatattgtgagggaaagagaattcactttggataatttanaaggttttrgagaagtgggagaatttttgcaataaaggtgttgggtaagtttaaacaatctaattcatgacwyaaataagagtatcagactagaatttta

SEQ ID NO: 36 - DNA, 201 bp, Pisum sativum
  source 1..201: mol_type = genomic DNA
  variation 101: note = n = a or g
atggtgcggcttcttactcaactckgaatgcacaragaacctacgttagttgagctttagaagttgmgcccgrtcttttcttcgayagtatcgactttctnggaagatccttcacaacaakcaatagtaagtggagtgatmatttcatccactaccactattgatcatcacctcwtccaacgataataccaagaacytgaa

SEQ ID NO: 37 - DNA, 201 bp, Pisum sativum
  source 1..201: mol_type = other DNA
  variation 101: note = n = t or c
gtcctgatgatccatcacctgstgatttttcttttggtatggttccacatarctatcctgatgcatatatgatgaagggtgataaaaaattctacagaagnggaccatggaatggtwtgcatgcaagtggttcaccacaagttaagccaaatccaatttatgattacaggtttgtttacaataaggatgaattttactata

SEQ ID NO: 38 - DNA, 201 bp, Pisum sativum
  source 1..201: mol_type = genomic DNA
  variation 101: note = n = a or g
  variation 101: note = n = a or g
gtatttttaaaggagctcgcattagcaaactacctcattcaccatctccaccaaaaagttcattcattgacgagatatcggtttctatgcacatatatatntcgaacagatcatcaattttgagggcraygataattgcgrttttcgarcgatttcgrctttgytcgrtaaaggagacaccatcaacttatccatgagttg

SEQ ID NO: 39 - DNA, 201 bp, Pisum sativum
  source 1..201: mol_type = genomic DNA
cttacaaacaccttacaaaactctttgttttttatcgaatgtcctcatgatgttgaccacaaattctttcaccagtccttcataacactgggataacccancaacagttttcattagtccaaaagttttaataaggtccatgacctctttgacctccacaacatctttgcccaattctctttccaccaccacccttctttg

SEQ ID NO: 40 - DNA, 201 bp, Pisum sativum
  source 1..201: mol_type = genomic DNA
  variation 101: note = n = g or a
atraaattcraagtgagctttcgagacttcaacgctcgacccacaccagttaccagagtaactctyaaaaacacattatccctctcttggaactcaagtgntttccttcgcttatcatgatagctcttctggagactytrcgrarctctcatcttctcttggatcactttgatattctytgtggtccaatctcaggcccaa

SEQ ID NO: 41 - DNA, 201 bp, Pisum sativum
  source 1..201: mol_type = genomic DNA
  variation 101: note = n = g or a
sgragctagggctccggtggtgtgttggcaaggttccaaccctttgatctggtccatggcttctaatctcatccattcaaattgaytaccacgcgtgtggnayaatmgactgaagaatatgtggaacrtgcgtttctaaccatctgatctgccatctcaattaatgagggagatcagatggctctccttttttagaatttc

SEQ ID NO: 42 - DNA, 201 bp, Pisum sativum
  source 1..201: mol_type = genomic DNA
  variation 101: note = n = c or t
akaaatttaggggtgttacattggccaccgcgatgaggggagtgaccaagwagcactagtctttaaaattactaatgttgtcggagtaaacttaaaacatnttttgaccaygcccaaggaraataaaccttgrccctrcgccaagccagttrattatcgttgagygttaaaaaggtataaaaagagtgtcaaggtcgacac

SEQ ID NO: 43 - DNA, 201 bp, Pisum sativum
  source 1..201: mol_type = genomic DNA
  variation 101: note = n = c or g
atcaaaaaacataaatgaagatgatgtcgattcaacgcagtatagaagactcattggatcactttgatatgtcacacaaggcctaatatarcatagtgtangtatggtgagaagattcatgcagaagctaaatgtatcacacctagcaactacggagaggatactaaggcatctgaaaggaactcttgacaatgaaattta

SEQ ID NO: 44 - DNA, 201 bp, Pisum sativum
  source 1..201: mol_type = genomic DNA
  variation 101: note = n = g or a
gccarcayttctgaaaccaagttmttatggtttgagctttcatatgatgcaagtatttggatccacttgagttcatytgctacatggtctggatgcaactntaactttgaacctgggtctaatgccttattcagggycaatcaagaartatgtcatctgatacttgggaagatcaagaagaagattgtgaagttgcttgct

SEQ ID NO: 45 - DNA, 201 bp, Pisum sativum
  source 1..201: mol_type = genomic DNA
  variation 101: note = n = t or c
ycraaycyggtctctcaymtwtaamtattaggttttatcattatttccytgttccttaggaacaaataaaggatgytggygactctgtcatttttccagcngcggcacattcagaaaagraaaacargcataagattgaaccaaattattcaaattgcaaaaaacaagaaatttyrggaagtgaagcaaagcaaaaacgga

SEQ ID NO: 46 - skipped

SEQ ID NO: 47 - DNA, 201 bp, Pisum sativum
  source 1..201: mol_type = genomic DNA
  variation 101: note = n = g or a
atgcaatgaaaaaggggaagtagagaartacaaagcaaggcatgtggctaaagggaactcacaagaacatgccatatattacaattargtttttgctcttntggmaagatgggatattatcaggactgtcttagcacttgcagcatgcaagaagtgacatgtatattagcttgaygtcaagagtgcattcytgcatggtga

SEQ ID NO: 48 - DNA, 201 bp, Pisum sativum
  source 1..201: mol_type = genomic DNA
  variation 101: note = n = c or t
tgaacctctgagtttccatctcccttgcttgcgtggtgctgagtgtgtcgcctgcgtgtgtgaatcattggcttggatttgcttgaccgttccacgcgtgntgttgactggtgatgtggctgccacatgttttaatgaaacacagcgtttcatgaacgcttttggagcctttgagtgtgggttcgagtcctggctggggcg

SEQ ID NO: 49 - DNA, 201 bp, Pisum sativum
  source 1..201: mol_type = genomic DNA
  variation 101: note = n = g or a
gtcacttcgatagctttgtcrcacaaggtctaacttagcatacagtgtaggtakgatgagtagattcatgcaaaagccaaaggtatcacatctagcagcgntgaagaggatactaaggtatctaaaaggaactcacractatggcattttgtttcctgcagctgatgaaggaaaataatrcaaattagtgggatacaccga

SEQ ID NO: 50 - DNA, 201 bp, Pisum sativum
  source 1..201: mol_type = genomic DNA
  variation 101: note = t or c
aggttgcttctgaacaaggctaggttttmtcagaggggtattaggagtgaaagttgagatgattgatgggtttttgatgtaagggtgattttgggttgganagggattacatgctctgcttcagaagtggaacatgtttggtgagaggattggattaaaggakagaagacttggatttgaatagcaaggataaggttgata

SEQ ID NO: 51 - DNA, 201 bp, Pisum sativum
  source 1..201: mol_type = genomic DNA
  variation 101: note = n = g or a
tgacttgacctcattgtgtttcatctrtrtaatgcttatgtgatttatttataggcgttatggctgctaagaaagatagattgaagcacgatagagttacncaacatacataggtttggaggtaaaaatctcaatcatcgtagacacatatcktttctagtccgrttgaggcgaagacgtcaatttctgggrctcatgcat

SEQ ID NO: 52 - DNA, 201 bp, Pisum sativum
  source 1..201: mol_type = genomic DNA
  variation 101: note = n = a or t
tatcagggcatgctgaacatgattatatgcacaacgaatggacgatttattgtcacataaaaaaawttcacaaggttaatamaatcatttacatctcttcntcctaaggggkttatttagcatgatascatccttgttataytttattgatgaatacaatatcraacaaaggcacactgaaatataacctaacaaataaga

SEQ ID NO: 53 - DNA, 201 bp, Pisum sativum
  source 1..201: mol_type = genomic DNA
  variation 101: note = n = a or g
caacattgtatttatattgcttgayraaagcttcgccaagatcattgaaggagmggatgtttgcactatccaaacccatataccatctragagcggcaccngacaggctgtcctggaaatagtggataaggagttgatcgttgtctrtctgagtcammatcttrcgtgcgtacatcacaagatggctgrgagggcaagtgt

SEQ ID NO: 54 - DNA, 201 bp, Pisum sativum
  source 1..201: mol_type = genomic DNA
  variation 101: note = n = t or c
aattycyaatcaacttttaagatgcatggttttatatcttcattctttaagtgyaatttatgtgtcaaaatttgaaagagtagttacctgatggatagggnttcttactagkactccatggttgcaatccattttcacaataagtctctatttgtatcttcaaaccattaacatcccaccatttcttccacctagcagtag

SEQ ID NO: 55 - DNA, 201 bp, Pisum sativum
  source 1..201: mol_type = genomic DNA
  variation 101: note = n = t or c
ccagaaagctagactccaatgacccctcttttcgtccaagctattatgttaagtggtttataaacgaaagagtgaatgaacgactaacccaagacgtgtgnctcgagagcatccattcgaagattcaaggaatgtgagaccccaagaatcttcttattttgtgtttgttaaaaaaagagtttaacgttgtgtcttaatagg

SEQ ID NO: 56 - DNA, 201 bp, Pisum sativum
  source 1..201: mol_type = genomic DNA
  variation 101: note = n = g or a
gagatgtttttggttggatgaygattactcggatagtcgagtraaacaactcgtatcctaataaccgagaaarggaatagaaractctaaaccgctctctntttcatctgaatatttatgaaaataaggttgtataagattgacgtattttagcatgaacracaaatacttgaacgactgagtaaaacaactcatatccaa

SEQ ID NO: 57 - DNA, 201 bp, Pisum sativum
  source 1..201: mol_type = genomic DNA
  variation 101: note = n = a or c
aaawtagttcattttaaatttgttgttmgaatcttayaatatttaaaacctgcccctgctacatacttattttattccgccaccactaatttaattttatntggttttgcagattctgattaggcagctttccctactttcraaaaatcaatcatcggatatgctgtttttctsggatcgcccctcatttcctggaaatca

SEQ ID NO: 58 - DNA, 201 bp, Pisum sativum
  source 1..201: mol_type = genomic DNA
  variation 101: note = n = a or c
aataataaaactttgggcgttacaactctcccccacttagaatattttcttcgtcgaaaatttaccygacgagaacaattttgggtatgtttcccgcatcnggctcttcagctcccaagtcatatttcctctaacyactcctccccaaacaactttctctagagaaatctctttgcctatcagcttcttcaattttcgatc

SEQ ID NO: 59 - DNA, 201 bp, Pisum sativum
  source 1..201: mol_type = genomic DNA
  variation 101: note = n = c or t
ttatcgtattttaggtcatgtcatttgcctcatgatagacttttcaaaatgtatcaattgtatctaattattactatttgcttcattcatgtctcaactgnacctttatctacttgcttcattcawggccataartatsttctctgtcctagacgactttagcagatatgtatgggatatattattttagtctaaagttga

SEQ ID NO: 60 - DNA, 201 bp, Pisum sativum
  source 1..201: mol_type = genomic DNA
  variation 101: note = n = c or t
attaacctaataataatatttattaagaaacaaaaataaagaaattaaataaakaaataaataaatagactagggggtgcatmattagttrtttgagtaantgggmtggctactgggtgtgtaaatagcraaggagagaggcccatatactttctraggcccayrttggaggggaagtccacacacacacacacaaagaga

SEQ ID NO: 61 - DNA, 201 bp, Pisum sativum
  source 1..201: mol_type = genomic DNA
  variation 101: note = n = g or t
ctctttaactcttcacattctttttmtaagtccaattgtkccccaatatcttcttcagygacttcatgctcttcaatgtgtaatttcatmcaaaacacatnaatagattctaatggaacatggtaaccttgtatttgaagtcytgcaacttcayacacacacaaggtaactcatgtgttrtcctaatraarcaaccacctg

SEQ ID NO: 62 - DNA, 201 bp, Pisum sativum
  source 1..201: mol_type = genomic DNA
  variation 101: note = n = t or c
atgcattggtttattgattgaagaattatgaataggtaatcatatgcaaagtaatcaacttttggacccctttgcttctaattctcaaccataatgacaancaaaatcctacaaagattcagatgacgatagtattcttgattgtcaccctctaacctctgaaacatgatgcaatgggatggatgatgcattgagattgag

SEQ ID NO: 63 - DNA, 201 bp, Pisum sativum
  source 1..201: mol_type = genomic DNA
  variation 101: note = n = g or a
gcatacattyagrgggagccttcatgraaacaygaaacacatmatctcaagttttkccatcatcawaaaagrkgagtatgtgagtgcaactttctgttagntgtattttgtatgatgtcaaaactaggatactttagcatttatgtatattggacagtatcctcttagtcttaatgtgcatcttagcattaggaagcataa

SEQ ID NO: 64 - DNA, 201 bp, Pisum sativum; identical to SEQ ID NO: 63
  source 1..201: mol_type = genomic DNA
  variation 101: note = n = t or a

SEQ ID NO: 65 - DNA, 201 bp, Pisum sativum
  source 1..201: mol_type = genomic DNA
  variation 101: note = n = t or c
tggaaccaaatactttatccctttggattctatgtatacttttgggycaataaccaatgccttcctttgaaccaagaratgttgctttggaaccaaacacntaattctccatgtttctagttataaamaatatartggggatgcctatgttcctccacrtcttagtttgtacctcttttactcttcrrttcaragttyact

SEQ ID NO: 66 - DNA, 201 bp, Pisum sativum
  source 1..201: mol_type = genomic DNA
  variation 101: note = n = g or a
atgggaggaaggaattgatgttgatgatgcgtacacaagtgataactttaaattgtgtgtcacgttgctttgcacaatcaattactttcctacatacrgtnatttgtctaggtacatcgtcaaggggyataaagcatgtccaatatgtgaagatgatacatgcttccaacacttaaaaaatggrgaaaaggttgtttacct

SEQ ID NO: 67 - DNA, 201 bp, Pisum sativum
  source 1..201: mol_type = genomic DNA
  variation 101: note = n = c or t
ttccccarcaaagtttccatmtgtcgmacctcgaaarataagaacataacttagcgaartgcartcgcacgctsgcatgatsgactaaacagagtcgccancgaactttatttrttcctaaaaakgawagaggaaatatcrataaaacccaagaaagaacgwcaatgattatggtcgtygcaaccaaatcaaggttcggga

SEQ ID NO: 68 - DNA, 201 bp, Pisum sativum
  source 1..201: mol_type = genomic DNA
  variation 101: note = n = c or t
tcgagtagagcgttgtcatcgttcaacgctcgtgatcgccgtggatctgcatcaaaggttttgatcgtcacaagagatctgcaccaaaggtttcaatcgtnataagaggtaaatattctwtcactgatcatgaccattcgtraggatctctaaaggagaaaattttaatttccgytgcgttttggaccgcaaatctccttc

SEQ ID NO: 69 - DNA, 201 bp, Pisum sativum
  source 1..201: mol_type = genomic DNA
  variation 101: note = n = t or c
agacttaatcctgygatgaaagaagtggtttgcaaaaaagttgtgaagytgttrgatgtgggtcttatttaccctatattcgatagctcatgggtgagtcncatacatgtagtacctaakaaggggagaacagtcgytrtcatgaataaaaaacatgagttgattcccacaagaaytgtcacgggttggagagtatgcayg

SEQ ID NO: 70 - DNA, 201 bp, Pisum sativum
  source 1..201: mol_type = genomic DNA
  variation 101: note = n = c or t
aacttcaactcgaaacttcaaacaaaccctaaaatttccagaccttcataaaacctcmcmaaatccaaaacaggccaacayaaacccaccctcaaatattnttctaaacacraaccctaaaccaaaatcatcaaaaactcgattaaaccaacatatcaaaacttcccaatytatgaaaccctaagttcycaagacctwaaa

SEQ ID NO: 71 - DNA, 201 bp, Pisum sativum
  source 1..201: mol_type = genomic DNA
  variation 101: note = n =g or a
agaagmagaaagatcattgcaacwacaacttgaacatctttcagaatttctcatgattagcgtagaagcggaatttggaacacaatrtkcagaaactgatnatgttgcacgtcataaactcakaatcagagctgrctattaaasctacacaataataaaccattagggtrccaaaattattctcacacaartacaacattg

SEQ ID NO: 72 - DNA, 201 bp, Pisum sativum
  source 1..201: mol_type = genomic DNA
  variation 101: note = n = t or a
ctaatatctaatacttatataaaayttttctctcatattttcataagarcatttgatgacttttgttgttcatcataacattcaatttctcgagtgaaacnttgrtttgtgtgagattttctaaaagcttcatcttttacctcaaacactaaataccattgatgagtataagcacgtmtcaactttaggagagagtgtaar

SEQ ID NO: 73 - DNA, 201 bp, Pisum sativum
  source 1..201: mol_type = genomic DNA
  variation 101: note = n = c or a
aggatcccctagcacaaaagcacacacacatcaaagagtcttatgaagcaaatcaagaatggacaagagttagtttagagatttggtccttctaatccatnttcaacattaggcattttactccaattttgcatagggaatatcctagaaactaagtccatttgtccatttmtttgcatttggtccataacaatcaaaaca

SEQ ID NO: 74 - DNA, 201 bp, Pisum sativum
  source 1..201: mol_type = genomic DNA
  variation 101: note = n = t or c
attcgatctttccattaacrgatcgattagacgattactatctaggatgcttccgcaaccgtygaaaacattttaaaaartgctaaagtttaaaactgatntattcaacccccmttctagatcggtactatcrtttaacatattcttttaccaatccatgcatattatgcatcactagagtttttttttggggttgatatt

SEQ ID NO: 75 - DNA, 201 bp, Pisum sativum
  source 1..201: mol_type = genomic DNA
  variation 101: note = n = t or a
ctcaaatgaaggattaacaagastgcccctaacaagttaagggtgggtcaccccaaggcaacrttgtgtrgggacatctactacaagatattttaccttgnctatttttttgcttgcctcygaacaaatgttgtttcaagcgttatgtgacytttcacttacacatgttctcctgatagaccaactaaggaaccttggaat

SEQ ID NO: 76 - DNA, 201 bp, Pisum sativum
  source 1..201: mol_type = genomic DNA
  variation 101: note = n = a or g
aattgttacctcttgtggttattgaaacctttgatgcagatataaggagtaatttctttaaaawtttytggattttagagtgtgtgtttctttattttttngtttacggttaggtgatgaaagcagtaaagtgaaaaaaktaaagaacaccacaagttatactagttccccttataaattgagagcatgtctagtccactt

SEQ ID NO: 77 - DNA, 201 bp, Pisum sativum
  source 1..201: mol_type = genomic DNA
  variation 101: note = n = g or a
tataatcatgtactccawgaacactccagtcrtaatakacacaccaaatgacatcactaaatactcatagtgaccatatctcattctgaatgtagtcttcnraatatcgtctgacttcacatgaatctgatgataaccaaaacacaaatcaatcttgttaaacacacaagcmccaaccaattgatccatcagatyatygat

SEQ ID NO: 78 - DNA, 201 bp, Pisum sativum
  source 1..201: mol_type = genomic DNA
  variation 101: note = n = c or t
gctcgacaacttgagtctgacctcaaactcttacgatcraagaratctttrtgcragaaacgcctagagcttcttaaggtcaagtatcttcagatcaaggncaaccttcctttctagtttttccttrtctattttgcatgtaatgataactttttctttgtaatgaatrttggccatttgggccttcggattyaatatagc

SEQ ID NO: 79 - DNA, 201 bp, Pisum sativum
  source 1..201: mol_type = genomic DNA
  variation 101: note = n = c or t
aacatggcaagtggggaagaaagacccgttaggaagtagttatttagttttactataaacaagggttgtaacttaggaraaggktgtgttggaastactgnaraactcacttactcaaagwatcagtgtcaaagaragaaaagagtramyttgagtgcaaaygtacgttcttataccattttatttatcaaaatatttact

SEQ ID NO: 80 - DNA, 201 bp, Pisum sativum
  source 1..201: mol_type = genomic DNA
  variation 101: note = n = t or c
gattgtcctccagtaaagcagaagttgcgcagaactcgacccgagatggccatgaaaatcaaagaggaggtacaaaagcagttggatgctggtttcctagntgtcactaattatctgccttgggtcgcgaacattgtgccggtaccgaagaaggatggaaaggtgaggatgtgtgtggactaccgggatttgaacaaagct

SEQ ID NO: 81 - DNA, 201 bp, Pisum sativum
  source 1..201: mol_type = genomic DNA
  variation 101: note = n = g or a
cttcagggttgataccccttttgccatctcgtagtctgagatcctgaaggtcattaaactttccgcttcccagctacattcgaacatttcaatgtttattngagccttcgagatcatatgttgggatctcattgttactcctatgggatgccaatttaccatcaacctcmttattgctctatgctaatgcaatattttttg

SEQ ID NO: 82 - DNA, 201 bp, Pisum sativum
  source 1..201: mol_type = genomic DNA
  variation 101: note = n = t or a
tggggaaaacagcgtggtgcarcatatctaatgaaaacagttacaacaaaaaaaactcaaaaacaacaaatyatgtaaatagagcttgaaaatgagtttanacagtccayaragatgcatctccggagkagttcatacaaaatycggagatgtrtccrratcaaaygaacgttttccagctaaaaaayargattaatgtga

SEQ ID NO: 83 - DNA, 201 bp, Pisum sativum
  source 1..201: mol_type = genomic DNA
  variation 101: note = n = t or g
agtcaatgataagattggcttcatagtcaaacacttcattctagaccaaagtcaactaccacatgacctatttttctatgatgaycatgatgaagaaaaanctcaccaatgtgtttaaagttcttgttatttcccgctttttcgcatttttcaattatgaaatttcaattcttgtaattccgtaaaattttgttcttgtat

SEQ ID NO: 84 - DNA, 201 bp, Pisum sativum
  source 1..201: mol_type = genomic DNA
  variation 101: note = n = c or a
tttcaaggtcaatagacactacccaaagctactacacgagaacccaactttggaagaagaaactgtagaagaactctctttrggaaaggctgcttatgcantcacttatctgccttgactcctcgggtgtgttctttcctttctcccactcttattttatatttatggtatttcattgaggacaatgtatgttttaagtgt

SEQ ID NO: 85 - DNA, 201 bp, Pisum sativum
  source 1..201: mol_type = genomic DNA
  variation 101: note = n = g or a
ggaggttggaactctgttccaarccttatctattgttgaagagaagaaaactrgggcacccatgtcttctttaagagatgcacaaaaggctattgaggctnacaayattgatsaatkgggtcgtatgatagagattgctgagaacaagaatarggctggattgggatttcaaccagggtcattcaatgtcagaactgaaga

SEQ ID NO: 86 - DNA, 201 bp, Pisum sativum
  source 1..201: mol_type = genomic DNA
  variation 101: note = n = a or g
acaatgatakctcatctgaattatgacacaastgtttgggtcatatgagtgaaaaggattgagaattttggcaaaaaagaatgtggtgtatggtgtttccnatgcaaagttaagaaagtgttcgcattktttggcggataagcaaagacaartttcctttatatcatccaacccaaagaagraatcagaagtattggattk

SEQ ID NO: 87 - DNA, 201 bp, Pisum sativum
  source 1..201: mol_type = genomic DNA
  variation 101: note = n = g or a
acatggtgaattctgacsttgaagttggaagaatcaaacatacttagaaattttctaagttaaaagtcaaatgaattctttttccaacttgaataactttnatatgagcttaaaattactttggttacttttacaatgttgtatctatttcaattctattaaattagatcacaaatttgatactatttggagcttgcatga

SEQ ID NO: 88 - DNA, 201 bp, Pisum sativum
  source 1..201: mol_type = genomic DNA
  variation 101: note = n = t or a
gtgaccataagtatcttggtcacttgatgaggcttgtctctactrctttgkagcttyagcctttcaacaagtacaagacctcaagcattaatcaggcatanaccatctttctcaccccsatagatcatcatctttgagaagttgcttcaataacttgtcaaacattgacaaggtttgcatgccatgagccttaagtaatat

SEQ ID NO: 89 - DNA, 201 bp, Pisum sativum
  source 1..201: mol_type = genomic DNA
  variation 101: note = n = t or c
ataatcctcctatcctcatgcctctagtcccaaggagaccgctgattatgtacttgacagtacttgacaattccatgggttgtgttctcggtcaacacgangagacaggtaggaaagagcatgccatatactacctgagtaagaaattcacagactgcgagtcaagatactcaatgcttgagagacaatacatgctgactc

SEQ ID NO: 90 - DNA, 201 bp, Pisum sativum
  source 1..201: mol_type = genomic DNA
  variation 101: note = n = c or t
wcataaatttgaacaacragtatatcattttttaatgacytacagaataaagttrtatcaaacttccctcgggtgaaatmattttctaaataaaaargtgnctagtctttcagaccatgctctargagcttgttttagaccatacaatgatttcttaagtttgaaaacaaaatctggatttttaggattttcaaaaccaga

SEQ ID NO: 91 - DNA, 201 bp, Pisum sativum
  source 1..201: mol_type = genomic DNA
  variation 101: note = n = c or g
aattgcaatccctaacaaaaatgaatttggatgcatgatttagccaacacaggacatgagctatggttaaagatgaacatgaaaatggaatcgcacatgtntcttggttggmtggttggattagagcaattatttgaggaatattcataaacataaacataagaaaaacatagaagtaggaaccacacaaatgtttgatat

SEQ ID NO: 92 - DNA, 201 bp, Pisum sativum
  source 1..201: mol_type = genomic DNA
  variation 101: note = n = c or t
  variation 101: note = n =c or t
atctcaatttcayyctcatttaaatcaacctcattcatcycracctcattgacttcaactyyattcatctcaactacaccctyatttaactyagyctmatncaccctaatatcattaactccaactacattcaactcaattacataacctgttttacctttgacaaattcytcatakakttttccaatcacatcttcttca

SEQ ID NO: 93 - DNA, 201 bp, Pisum sativum
  source 1..201: mol_type = genomic DNA
  variation 101: note = n = t or c
caagaagtggaactctttgatgtctggggaatagatttcatgggaycgtttccatcgtcaatgggaaacaaatacatcttagtagttgttgactacgtctntaagtggattgaggttgtagcstcacctaccaacaacactcgtgtggtyatcaaattattcaaaaayaacatatttcctagatttggartacctcgcctc

SEQ ID NO: 94 - DNA, 201 bp, Pisum sativum
  source 1..201: mol_type = genomic DNA
  variation 101: note = n = a or g
agggctgaaaaagcaaactcgattacaggatgggcattygattccgtaaggaaatacgaatcttactcgactggggaagaaaaaagacttcgactgaaranygcatgagatatattatctattaccgtcagaacgtagataacatattcgcatggaagattatccacaaccggttactgggttaataaaggataaatcgac

SEQ ID NO: 95 - DNA, 201 bp, Pisum sativum
  source 1..201: mol_type = genomic DNA
  variation 101: note = n = a or t
caggagagacatgaaccatctgagcaaaagtgggagacaacacctgatagccccacccttaccatgcctactgtggatagcatagtaagtgttagctaacngagtagggactggattccctccgatgaagatgcagactgcagcatagtcaataaaattaggcatactaggaaacagaacgatcccatagatcataacagc

SEQ ID NO: 96 - DNA, 201 bp, Pisum sativum
  source 1..201: mol_type = genomic DNA
  variation 101: note = n = t or g
attcacccccyattctaaccattacaaaacttrggaagacrrgtttgtgagactgaatgggagaaattrtgcgtccaaggttaccatcgrrgacgmaaatncstaktttttccctttatattggacaraggatcctttggctataaayaactttgactttgaatacctaaccatcacacacacacacacacacacacacac

SEQ ID NO: 97 - DNA, 202 bp, Pisum sativum
  source 1..202: mol_type = genomic DNA
  variation 101: note = n = c or a
ytgataaaggytgmtgggttgttgaakactgtggttgggttctctcagtgctatgagggtctarttaaggaattcattgtcaamattcytraggatattgcatgataagaacaayaaggaattttgcaaggtgtttgtgagaggtaagtgtatcacattctctcccactgttattaataattttykgggaagaaaasttgag

SEQ ID NO: 98 - DNA, 201 bp, Pisum sativum
  source 1..201: mol_type = genomic DNA
  variation 101: note = n = a or t
aaaccttccatttatgggcttaacaatcaattatataggttgtytaattgattatgacattgaataagcatgtgaattgtttccaawtttatacaycgccntggmyaayaaatagaatgrttttccatcaccttttcatatccataaaargagaataaatctgacttttcatttctttcaccatctttgtttggtttggag

SEQ ID NO: 99 - DNA, 201 bp, Pisum sativum
  source 1..201: mol_type = genomic DNA
  variation 101: note = n = c or t
tgagcacaaggtcaccttctctgaatacacgaggyctgaccttcttatcaaaagctttcttcattctctgmtgatatagctgaccatggcayrtggcartnaaccttttctmttcaatcaaattcagctgaacgtacctggtctgacacyattcaacttctatcaacttggcttccatcaagacayrcaatgatgggattt

SEQ ID NO: 100 - DNA, 201 bp, Pisum sativum
  source 1..201: mol_type = genomic DNA
  variation 101: note = n = a or g
gttggaattccagtgtgctgaggaattcgagcgtgatgcgctcgtatgtcggcgcttccaggctcatgaactctagcattcctaaaacgyggaacatccgntatacctccattttgagccytagtgcgttcagagtatgcycacacatgtaycttgtcgrtgtgagttttcgcttccggtgaatttgatacctcttttctt

SEQ ID NO: 101 - DNA, 201 bp, Pisum sativum
  source 1..201: mol_type = genomic DNA
  variation 101: note = n = a or g
cccgcggtctcgaaaccctaagatggggatggcttcttcctacttcctagttaccaccaccagacttgaagcattttgtgatggatgcttttaattttttnttcctagctaagcgatcaaccgttaataagagagagagcaaggtaagagatgatattggagttgatttgtggtgacttcagcaagtggcttaggcattat

SEQ ID NO: 102 - DNA, 201 bp, Pisum sativum
  source 1..201: mol_type = genomic DNA
  variation 101: note = n = t or c
cctagtcaaacaaytacttrtccacgrcmcacaccgaggtatcattgtgtacaagcatttccatttaagttattcgtcaaaccctaattatcttcctaatncattcaattagttttcttctaaggtttcctcaccaatcattacttycaawcatattatcacattcatacaacaattaagtcataacatamtcatcatgct

SEQ ID NO: 103 - DNA, 201 bp, Pisum sativum
  source 1..201: mol_type = genomic DNA
  variation 101: note = n = g or c
caaaatgccatgcgtgcgcctatgtggacctatcacatgctaaccctaactaaaacactttcagcaacagaaaagcgttcttcatggattaaaagcgtggnctaaagtagcagctcgtcttcttcctcgcgccatgcatgaacagtggatgcatcttcatgcatcaagaacttttgttccagaaattaaaattaagcatat

SEQ ID NO: 104 - DNA, 201 bp, Pisum sativum
  source 1..201: mol_type = genomic DNA
  variation 101: note = n = t or g
ccatgttataatatgaaatgcacaaatgaacataaacattaagctcttagaaactcactcatggaaagtccaaaaaaataakgtgagtaatggttggaaancccttgaaataaggaacaaaagtcatgttrkgaaaaaattcatttggagtttagaaatttatgaaaactggctgtgaargtttgggtacaaaacatrtct

SEQ ID NO: 105 - DNA, 201 bp, Pisum sativum
  source 1..201: mol_type = genomic DNA
  variation 101: note = n = g or a
tgtaygctagttgtattgaatcctcgttcacataaaaatttaacataatccactttatcattatgttagaatgaatagctttgactaggtcaatatgatcngctccatatgcaaattcatcatctgcastattttttgaaatgatatgtgmagctacaacacaacaaatatmaaaaaatatttayattaaattaaaacata

SEQ ID NO: 106 - DNA, 201 bp, Pisum sativum
  source 1..201: mol_type = genomic DNA
  variation 101: note = n = c or t
gtaagaaactttgggaaaactaacaagagakgacccataaagtgggtacctaaggataaaataacttatgttgcagacatccttatcagctcagttgaaanaccrgtcatggtacctgaacaatggattctcgcaacacataacatgaaraaggtatatgttccaagatttggaacttaagcctggaggcttcattggttt

SEQ ID NO: 107 - DNA, 201 bp, Pisum sativum
  source 1..201: mol_type = genomic DNA
  variation 101: note = n = a or g
gttgcctacatatcaccacggttggaatttccaaccatggtgaaatgtaacacactatctagtttttcacaatggaccttaactcgtggtggaaagtaccncacttatgaccaccctctaacttaccatggttcgtcaatcgtgatggtatcccttccaatcatgttgtgaaagggccattacatagtagtgtgtaattct

SEQ ID NO: 108 - DNA, 201 bp, Pisum sativum
  source 1..201: mol_type = genomic DNA
  variation 101: note = n = t or c
gatgctgagcagttgcgttcatcrccaaatgaggacgactctgattgggaggatgaagaccctgatgacgaaggtatcatttatgtggaatagctgtcccngaaagcatcagtgttggtaagtatgttttgatgagcttatgtcatgaagatgattagttcagttatactttgtatatttgagtttggttygctttagaat

SEQ ID NO: 109 - DNA, 201 bp, Pisum sativum
  source 1..201: mol_type = genomic DNA
  variation 101: note = n = a or g
gattggatcatacccccagcagaggtgaaccgttgttcaacatctgtatggcacgtttgctgcagttgctcttgatagcattcatgattggtactccccanagaggtttatttcctcacccgtcagtgaaagcaaagcttgacttccccatagtagtccccggaaagggtctggccttgtcttgacatatagagatgtcat

SEQ ID NO: 110 - DNA, 201 bp, Pisum sativum
  source 1..201: mol_type = genomic DNA
  variation 101: note = n = c or a
tttccaactaacataacattccaactaactgagtaaatattaactaactgagttatyagttaactcagtgagtcatccmyaactaactccaagccaccctnaactaattcctaacctmattccaaagmtaacactttccaaacctaakctttatttaagaaattcatcattcacaattttaggacccttgaaaaccctgtg

SEQ ID NO: 111 - DNA, 201 bp, Pisum sativum
  source 1..201: mol_type = genomic DNA
  variation 101: note = n = a or t
tgaggtgaatttgtttagcatgctagtgactagaatcagaatcttttactctaatatacaattttttgccccacatagaaagcttctttgaattatagcantgctgcaaaaacagcccatagtattaaagttgcaataagtgatatttctccttacctgtgtcaggataattgagtaatgtctttttgtcatatatttgca

SEQ ID NO: 112 - DNA, 201 bp, Pisum sativum
  source 1..201: mol_type = genomic DNA
  variation 101: note = n = g or t
tttatttaagagtggttacarctaagagagagcaacaatgtgattratggataaattgacatcaytgwcgatttttaggcaatgtgatgatttggcacgtngctcgaagtcgaaccaaatttrtgcattttttgtcttttttgcaacggttcaycactacaaataatacatttcatgacaaagctttcacttcaaccaatt

SEQ ID NO: 113 - DNA, 201 bp, Pisum sativum
  source 1..201: mol_type = genomic DNA
  variation 101: note = n = a or g
caaaggttgagcagtgtcttgattgtaggggtatattaccatcatcatggttatgtcatctttaagggctccattgtgcatgctccagttcctcaggattngggttttgacctctagtcaaccctaatcaattgcattcttccaatcagggattttcaaggagatgaggtatttttatggaatgaggatcacatgatcatt

SEQ ID NO: 114 - DNA, 201 bp, Pisum sativum
  source 1..201: mol_type = genomic DNA
  variation 101: note = n = g or a
tgagagaggagggycccttttgcacgtactatcataattgattaatatagtasggtgttgactcaagataaccccayagatcaaakaaggaamagytattnccattttcacagcataagaggcaacatgcttcatagtctgataaaaaacataggatcmaaaacaaaatttgactcrgtgccaacaatatagataarctta

SEQ ID NO: 115 - DNA, 201 bp, Pisum sativum
  source 1..201: mol_type = genomic DNA
  variation 101: note = n = c or t
tgcttaatcccacraaaagagacttytgctccrccctcaagcatgtgaattcaatgctcaatctatccataaagrgacttctgctctgcctacaagcacgngacttcaatgcctgaacaacccgttcaggacttccttctctgcctgtaagcatgagacttcactgctcaatacwcagaaagatacttcttcrctcaagaa

SEQ ID NO: 116 - DNA, 201 bp, Pisum sativum
  source 1..201: mol_type = genomic DNA
  variation 101: note = n = c or t
gagccattggatgcattttcgagatctaatcgtgggccatcaatcatatgacttattttaatgcctcgtgtgtctcatttactaaggcttatggtgagcgngcgcatgtggagcgtttgattctccaygtcaattaatgaaatctcatccaackcctctccttttttctgattttctgaatttccattttattttctttaa

SEQ ID NO: 117 - DNA, 201 bp, Pisum sativum
  source 1..201: mol_type = genomic DNA
  variation 101: note = n = a or g
ataacactcgtgtaccaatgyacataccaaatagaaraaaagtttaaagaaaaaaagtargatttgrtacataccatacaagtttcacacacataccggtngcargtacatacccgatactgatactttgtctaaaatgacctatcaatgyttcacatrttctcacccattatgcatgtttcaaacttccacgataaattt

SEQ ID NO: 118 - DNA, 201 bp, Pisum sativum
  source 1..201: mol_type = genomic DNA
  variation 101: note = n = g or c
tgataataaagatcccaattctagttttagaattgggggcagacgtaccctaagcgaggacgaaaggggaacygcctaaacaaatctggtgttgttttctntttctcytaactctttaaattctgcattaattacgttttrtgtgaaattaatagcataataaatctcgcttaattgytgttcatagtagctgttcgataa

SEQ ID NO: 119 - DNA, 201 bp, Pisum sativum
  source 1..201: mol_type = genomic DNA
  variation 101: note = n = g or a
agcactcttaccgaacagatcctttcccctcaaggttttcaactcctttcgcagctcaaggaattggtctttcatttcatccatcttctcataaacatccngaccttcagatggctcgaaatgatagatggtgtcctcaacgcggggcaaagtatgaataactgttggaggcacagacatgatygggctagatgtcggcat

SEQ ID NO: 120 - DNA, 201 bp, Pisum sativum
  source 1..201: mol_type = genomic DNA
  variation 101: note = n = g or a
ttttgggtgataaattttttgttttaggaatcaataatgtcgycgaagcgaattttcaaggggaarcaaacagaagcagaatyatcccgtcctcggaaacngaccatccgtcatctgatttcgcatgatatcatctttgataacccaragcatgaacgaaggtastcttctcacgtcaaacgggagataactcygacaagg

SEQ ID NO: 121 - DNA, 201 bp, Pisum sativum
  source 1..201: mol_type = genomic DNA
  variation 101: note = n = a or g
aaattggtagcgccgactcaagtttttaattgggatctattcaacccccccccccccttttagatccgtgccatagtctaacacccttgatatacaatcanaagggtagacaaaatacaacacaaaaggactytttaagacttgagagtttctaagaatatacaagtgttaagaaattctaagttaaacttgtgwtttttg

SEQ ID NO: 122 - DNA, 201 bp, Pisum sativum
  source 1..201: mol_type = genomic DNA
  variation 101: note = n = c or t
tcaatcgtccctcactggcaccttcttctaatctcaaamccatgtttaccatctcgacaaaatcactaggagcgtttgcaaccatcctgtcataatagaangggctyagagtcttcaaaaatagctttgtcatttacttctcttctaacgrtggactaacstgcccaacaatttygcaymacctytgtrtgtactccttgm

SEQ ID NO: 123 - DNA, 201 bp, Pisum sativum
  source 1..201: mol_type = genomic DNA
  variation 101: note = n = t or g
tgcayatatatatacmttgttcgagcttctccaagtcttccaagtccttttcawtatccactttcaaagggggagatcttaamcaattttgtgcacatatnaaagcttcaacaatgtatggtgtaagagaaatcctataacaactaagaactctaccccctgtgctaaaagcagactctraagyaacagtagatattggca

SEQ ID NO: 124 - DNA, 201 bp, Pisum sativum
  source 1..201: mol_type = genomic DNA
  variation 101: note = n = a or g
arattakgatkatttttrgttatttkctttttttaaygycatgtttcttttcatgatttcatatgcttatgattctcaatatgagcatgccccmtgattanttagttgatcaaagttatgtttgatcaagtgattacacttgtccaygacttrycttgaacatttrcwtgcttcctctatmttgtcaagtgatcataagtc